European Patent Specification EP 3 870 288 B1, published December 11, 2024. Title: Pan-ELR+ CXC Chemokine Antibodies for the Treatment of Hidradenitis Suppurativa. Applicant: ELI LILLY AND COMPANY. The sequence listing filed with the application follows.

SEQUENCE LISTING (19 sequences)

SEQ ID NO: 1 - protein, 452 aa, Artificial Sequence
  synthetic construct
QVQLVQSGAEVKKPGASVKVSCKASGYEFTSYWIHWVRQAPGQGLEWMGNISPNSGSANYNEKFKSRVTMTRDTSTSTVYMELSSLRSEDTAVYYCAREGPYSYYPSREYYGSDLWGQGTLVTVSSASTKGPSVFPLAPCSRSTSESTAALGCLVKDYFPEPVTVSWNSGALTSGVHTFPAVLQSSGLYSLSSVVTVPSSSLGTKTYTCNVDHKPSNTKVDKRVESKYGPPCPPCPAPEFLGGPSVFLFPPKPKDTLMISRTPEVTCVVVDVSQEDPEVQFNWYVDGVEVHNAKTKPREEQFNSTYRVVSVLTVLHQDWLNGKEYKCKVSNKGLPSSIEKTISKAKGQPREPQVYTLPPSQEEMTKNQVSLTCLVKGFYPSDIAVEWESNGQPENNYKTTPPVLDSDGSFFLYSRLTVDKSRWQEGNVFSCSVMHEALHNHYTQKSLSLSLG

SEQ ID NO: 2 - protein, 126 aa, Artificial Sequence
  synthetic construct
QVQLVQSGAEVKKPGASVKVSCKASGYEFTSYWIHWVRQAPGQGLEWMGNISPNSGSANYNEKFKSRVTMTRDTSTSTVYMELSSLRSEDTAVYYCAREGPYSYYPSREYYGSDLWGQGTLVTVSS

SEQ ID NO: 3 - protein, 214 aa, Artificial Sequence
  synthetic construct
EIVLTQSPATLSLSPGERATLSCRASQSISNNLHWYQQKPGQAPRLLIYYTSRSVSGIPARFSGSGSGTDFTLTISSLEPEDFAVYYCGQNNEWPEVFGGGTKVEIKRTVAAPSVFIFPPSDEQLKSGTASVVCLLNNFYPREAKVQWKVDNALQSGNSQESVTEQDSKDSTYSLSSTLTLSKADYEKHKVYACEVTHQGLSSPVTKSFNRGEC

SEQ ID NO: 4 - protein, 107 aa, Artificial Sequence
  synthetic construct
EIVLTQSPATLSLSPGERATLSCRASQSISNNLHWYQQKPGQAPRLLIYYTSRSVSGIPARFSGSGSGTDFTLTISSLEPEDFAVYYCGQNNEWPEVFGGGTKVEIK

SEQ ID NO: 5 - DNA, 1356 bp, Artificial Sequence
  synthetic construct
caggtgcagctggtgcagtctggtgctgaagtgaagaagcctggggcctcagtgaaggtgtcctgcaaggcatctggctacgagttcaccagctactggattcactgggtgcgacaggcccctggacaagggcttgagtggatgggaaatatttctcctaatagtggtagtgctaactacaatgagaagttcaagagcagagtcaccatgaccagggacacgtccacgagcacagtctacatggagctgagcagcctgagatctgaggacacggccgtgtattactgtgcgagagagggcccttacagttattatccgagtagggagtactatggctctgacctctgggggcaagggaccctagtcacagtctcctcagcctccaccaagggcccatcggtcttcccgctagcgccctgctccaggagcacctccgagagcacagccgccctgggctgcctggtcaaggactacttccccgaaccggtgacggtgtcgtggaactcaggcgccctgaccagcggcgtgcacaccttcccggctgtcctacagtcctcaggactctactccctcagcagcgtggtgaccgtgccctccagcagcttgggcacgaagacctacacctgcaacgtagatcacaagcccagcaacaccaaggtggacaagagagttgagtccaaatatggtcccccatgcccaccctgcccagcacctgagttcctggggggaccatcagtcttcctgttccccccaaaacccaaggacactctcatgatctcccggacccctgaggtcacgtgcgtggtggtggacgtgagccaggaagaccccgaggtccagttcaactggtacgtggatggcgtggaggtgcataatgccaagacaaagccgcgggaggagcagttcaacagcacgtaccgtgtggtcagcgtcctcaccgtcctgcaccaggactggctgaacggcaaggagtacaagtgcaaggtctccaacaaaggcctcccgtcctccatcgagaaaaccatctccaaagccaaagggcagccccgagagccacaggtgtacaccctgcccccatcccaggaggagatgaccaagaaccaggtcagcctgacctgcctggtcaaaggcttctaccccagcgacatcgccgtggagtgggaaagcaatgggcagccggagaacaactacaagaccacgcctcccgtgctggactccgacggctccttcttcctctacagcaggctaaccgtggacaagagcaggtggcaggaggggaatgtcttctcatgctccgtgatgcatgaggctctgcacaaccactacacacagaagagcctctccctgtctctgggt

SEQ ID NO: 6 - DNA, 642 bp, Artificial Sequence
  synthetic construct
gaaattgtgttgacacagtctccagccaccctgtctttgtctccaggggaaagagccaccctctcctgcagggccagtcaaagtatcagcaataacctacactggtaccaacagaaacctggccaggctcccaggctcctcatctattatacttcccggtccgtctctggcatcccagccaggttcagtggcagtgggtctgggacagacttcactctcaccatcagcagcctagagcctgaagattttgcagtttattactgtggacagaataacgagtggcctgaggtgttcggcggagggaccaaggtggagatcaaacgaactgtggctgcaccatctgtcttcatcttcccgccatctgatgagcagttgaaatctggaactgcctctgttgtgtgcctgctgaataacttctatcccagagaggccaaagtacagtggaaggtggataacgccctccaatcgggtaactcccaggagagtgtcacagagcaggacagcaaggacagcacctacagcctcagcagcaccctgacgctgagcaaagcagactacgagaaacacaaagtctacgcctgcgaagtcacccatcagggcctgagctcgcccgtcacaaagagcttcaacaggggagagtgc

SEQ ID NO: 7 - protein, 11 aa, Artificial Sequence
  synthetic construct
RASQSISNNLH

SEQ ID NO: 8 - protein, 7 aa, Artificial Sequence
  synthetic construct
YTSRSVS

SEQ ID NO: 9 - protein, 9 aa, Artificial Sequence
  synthetic construct
GQNNEWPEV

SEQ ID NO: 10 - protein, 10 aa, Artificial Sequence
  synthetic construct
GYEFTSYWIH

SEQ ID NO: 11 - protein, 17 aa, Artificial Sequence
  synthetic construct
NISPNSGSANYNEKFKS

SEQ ID NO: 12 - protein, 17 aa, Artificial Sequence
  synthetic construct
EGPYSYYPSREYYGSDL

SEQ ID NO: 13 - protein, 73 aa, Homo sapiens
ASVATELRCQCLQTLQGIHPKNIQSVNVKSPGPHCAQTEVIATLKNGRKACLNPASPIVKKIIEKMLNSDKSN

SEQ ID NO: 14 - protein, 73 aa, Homo sapiens
APLATELRCQCLQTLQGIHLKNIQSVKVKSPGPHCAQTEVIATLKNGQKACLNPASPMVKKIIEKMLKNGKSN

SEQ ID NO: 15 - protein, 73 aa, Homo sapiens
ASVVTELRCQCLQTLQGIHLKNIQSVNVRSPGPHCAQTEVIATLKNGKKACLNPASPMVQKIIEKILNKGSTN

SEQ ID NO: 16 - protein, 74 aa, Homo sapiens
AAVLRELRCVCLQTTQGVHPKMISNLQVFAIGPQCSKVEVVASLKNGKEICLDPEAPFLKKVIQKILDGGNKEN

SEQ ID NO: 17 - protein, 75 aa, Homo sapiens
VSAVLTELRCTCLRVTLRVNPKTIGKLQVFPAGPQCSKVEVVASLKNGKQVCLDPEAPFLKKVIQKILDSGNKKN

SEQ ID NO: 18 - protein, 70 aa, Homo sapiens
AELRCMCIKTTSGIHPKNIQSLEVIGKGTHCNQVEVIATLKDGRKICLDPDAPRIKKIVQKKLAGDESAD

SEQ ID NO: 19 - protein, 72 aa, Homo sapiens
SAKELRCQCIKTYSKPFHPKFIKELRVIESGPHCANTEIIVKLSDGRELCLDPKENWVQRVVEKFLKRAENS